European Patent Specification EP 3 649 153 B1, published June 11, 2025. Title: COMPOUNDS AND METHODS FOR TUMOUR-SPECIFIC CELL DEPLETION. Applicant: TUSK THERAPEUTICS LTD CANCER RESEARCH TECHNOLOGY LIMITED. The sequence listing filed with the application follows.

SEQUENCE LISTING (4 sequences)

SEQ ID NO: 1 - protein, 272 aa, homo sapiens
MDSYLLMWGLLTFIMVPGCQAELCDDDPPEIPHATFKAMAYKEGTMLNCECKRGFRRIKSGSLYMLCTGNSSHSSWDNQCQCTSSATRNTTKQVTPQPEEQKERKTTEMQSPMQPVDQASLPGHCREPPPWENEATERIYHFVVGQMVYYQCVQGYRALHRGPAESVCKMTHGKTRWTQPQLICTGEMETSQFPGEEKPQASPEGRPESETSCLVTTTDFQIQTEMAATMETSIFTTEYQVAVAGCVFLLISVLLLSGLTWQRRQRKSRRTI

SEQ ID NO: 2 - protein, 222 aa, homo sapiens
CQAELCDDDPPEIPHATFKAMAYKEGTMLNCECKRGFRRIKSGSLYMLCTGNSSHSSWDNQCQCTSSATRNTTKQVTPQPEEQKERKTTEMQSPMQPVDQASLPGHCREPPPWENEATERIYHFVVGQMVYYQCVQGYRALHRGPAESVCKMTHGKTRWTQPQLICTGEMETSQFPGEEKPQASPEGRPESETSCLVTTTDFQIQTEMAATMETSIFTTEYQ

SEQ ID NO: 3 - protein, 139 aa, murine
METDTLLLWVLLLWVPGSTGEVQLQQSGAELVRPGTSVKLSCKVSGDTITAYYIHFVKQRPGQGLEWIGRIDPEDDSTEYAEKFKNKATITANTSSNTAHLKYSRLTSEDTATYFCTTDNMGATEFVYWGQGTLVTVSS

SEQ ID NO: 4 - protein, 129 aa, murine
METDTLLLWVLLLWVPGSTGQVVLTQPKSVSASLESTVKLSCKLNSGNIGSYYMHWYQQREGRSPTNLIYRDDKRPDGAPDRFSGSIDISSNSAFLTINNVQTEDEAMYFCHSYDGRMYIFGGGTKLTV